European Patent Application EP 4 806 460 A1, published September 16, 2026. Title: Vaccine composition for inducing anti-IgE antibody. Applicant: 株式会社ファンペップ. The sequence listing filed with the application follows.

SEQUENCE LISTING (39 sequences)

SEQ ID NO: 1 - protein, 20 aa, synthetic construct
  source 1..20: note = Artificial T helper cell epitope (AJP001)
ELKLIFLHRLKRLRKRLKRK

SEQ ID NO: 2 - protein, 14 aa, synthetic construct
EDSTKKCADSNPRG

SEQ ID NO: 3 - protein, 14 aa, synthetic construct
DSTKKCADSNPRGV

SEQ ID NO: 4 - protein, 14 aa, synthetic construct
STKKCADSNPRGVS

SEQ ID NO: 5 - protein, 18 aa, synthetic construct
GHTFEDSTKKCADSNPRG

SEQ ID NO: 6 - protein, 18 aa, synthetic construct
HTFEDSTKKCADSNPRGV

SEQ ID NO: 7 - protein, 18 aa, synthetic construct
TFEDSTKKCADSNPRGVS

SEQ ID NO: 8 - protein, 14 aa, synthetic construct
KSPTITCLVVDLAP

SEQ ID NO: 9 - protein, 14 aa, synthetic construct
SPTITCLVVDLAPS

SEQ ID NO: 10 - protein, 14 aa, synthetic construct
PTITCLVVDLAPSK

SEQ ID NO: 11 - protein, 18 aa, synthetic construct
LFIRKSPTITCLVVDLAP

SEQ ID NO: 12 - protein, 18 aa, synthetic construct
FIRKSPTITCLVVDLAPS

SEQ ID NO: 13 - protein, 18 aa, synthetic construct
IRKSPTITCLVVDLAPSK

SEQ ID NO: 14 - protein, 14 aa, synthetic construct
HSTRKEEKQRNGTL

SEQ ID NO: 15 - protein, 14 aa, synthetic construct
STRKEEKQRNGTLT

SEQ ID NO: 16 - protein, 14 aa, synthetic construct
NHSTRKEEKQRNGT

SEQ ID NO: 17 - protein, 15 aa, synthetic construct
VNHSTRKEEKQRNGT

SEQ ID NO: 18 - protein, 16 aa, synthetic construct
PVNHSTRKEEKQRNGT

SEQ ID NO: 19 - protein, 17 aa, synthetic construct
KPVNHSTRKEEKQRNGT

SEQ ID NO: 20 - protein, 18 aa, synthetic construct
GKPVNHSTRKEEKQRNGT

SEQ ID NO: 21 - protein, 19 aa, synthetic construct
SGKPVNHSTRKEEKQRNGT

SEQ ID NO: 22 - protein, 20 aa, synthetic construct
ASGKPVNHSTRKEEKQRNGT

SEQ ID NO: 23 - protein, 23 aa, synthetic construct
WSRASGKPVNHSTRKEEKQRNGT

SEQ ID NO: 24 - protein, 25 aa, synthetic construct
LTWSRASGKPVNHSTRKEEKQRNGT

SEQ ID NO: 25 - protein, 28 aa, synthetic construct
TVNLTWSRASGKPVNHSTRKEEKQRNGT

SEQ ID NO: 26 - protein, 30 aa, synthetic construct
KGTVNLTWSRASGKPVNHSTRKEEKQRNGT

SEQ ID NO: 27 - protein, 18 aa, synthetic construct
KPVNHSTRKEEKQRNGTL

SEQ ID NO: 28 - protein, 18 aa, synthetic construct
PVNHSTRKEEKQRNGTLT

SEQ ID NO: 29 - protein, 14 aa, synthetic construct
ETYQCRVTHPHLPR

SEQ ID NO: 30 - protein, 14 aa, synthetic construct
TYQCRVTHPHLPRA

SEQ ID NO: 31 - protein, 14 aa, synthetic construct
YQCRVTHPHLPRAL

SEQ ID NO: 32 - protein, 18 aa, synthetic construct
WIEGETYQCRVTHPHLPR

SEQ ID NO: 33 - protein, 18 aa, synthetic construct
IEGETYQCRVTHPHLPRA

SEQ ID NO: 34 - protein, 18 aa, synthetic construct
EGETYQCRVTHPHLPRAL

SEQ ID NO: 35 - protein, 19 aa, synthetic construct
  source 1..19: note = Artificial T helper cell epitope (UBITh1)
ISITEIKGVIVHRIETILF

SEQ ID NO: 36 - protein, 18 aa, synthetic construct
  source 1..18: note = Artificial T helper cell epitope (UBITh2)
KKKIITITRIITIITTID

SEQ ID NO: 37 - protein, 19 aa, synthetic construct
  source 1..19: note = Artificial T helper cell epitope (UBITh3)
ISISEIKGVIVHKIETILF

SEQ ID NO: 38 - protein, 19 aa, synthetic construct
  source 1..19: note = Artificial T helper cell epitope
ISITEIRTVIVTRIETILF

SEQ ID NO: 39 - protein, 14 aa, synthetic construct
  source 1..14: note = Artificial T helper cell epitope (Tetanous toxisoid peptide)
QYIKANSKFIGITE